European Patent Application EP 4 810 515 A1, published September 23, 2026. Title: GDF15中和抗体及其用途. Applicant: 上海海路生物技术有限公司. Application CN. The sequence listing filed with the application follows.

SEQUENCE LISTING (229 sequences)

SEQ ID NO: 1 - protein, 7 aa, synthetic construct
TYGIGVG

SEQ ID NO: 2 - protein, 16 aa, synthetic construct
HIWWNNNKYFNTALKS

SEQ ID NO: 3 - protein, 8 aa, synthetic construct
MGYDIMDY

SEQ ID NO: 4 - protein, 7 aa, synthetic construct
ISGMGVS

SEQ ID NO: 5 - protein, 16 aa, synthetic construct
HIYWDDDKRYNPSLKS

SEQ ID NO: 6 - protein, 8 aa, synthetic construct
AGWDFFDY

SEQ ID NO: 7 - protein, 7 aa, synthetic construct
TSGMGVS

SEQ ID NO: 8 - protein, 8 aa, synthetic construct
TGWDFFDY

SEQ ID NO: 9 - protein, 5 aa, synthetic construct
DYNLN

SEQ ID NO: 10 - protein, 17 aa, synthetic construct
DLNPYNGGIIYNQKFKG

SEQ ID NO: 11 - protein, 10 aa, synthetic construct
EGRGGAWFDS

SEQ ID NO: 12 - protein, 5 aa, synthetic construct
DYNMN

SEQ ID NO: 13 - protein, 17 aa, synthetic construct
LINPYNGGTRYNQNFKG

SEQ ID NO: 14 - protein, 10 aa, synthetic construct
EVRLGNALDY

SEQ ID NO: 15 - protein, 5 aa, synthetic construct
GYNMN

SEQ ID NO: 16 - protein, 17 aa, synthetic construct
LINPSNGGSSYSQKFKG

SEQ ID NO: 17 - protein, 16 aa, synthetic construct
HIWWNDNKYYNTALKS

SEQ ID NO: 18 - protein, 8 aa, synthetic construct
LAYDYVDS

SEQ ID NO: 19 - protein, 17 aa, synthetic construct
LINPYNGGTIYNQKFKG

SEQ ID NO: 20 - protein, 10 aa, synthetic construct
EVRLGNAMDY

SEQ ID NO: 21 - protein, 16 aa, synthetic construct
HIYWDDDKRYKPSLKS

SEQ ID NO: 22 - protein, 8 aa, synthetic construct
SAYGMTDY

SEQ ID NO: 23 - protein, 5 aa, synthetic construct
NYDIN

SEQ ID NO: 24 - protein, 17 aa, synthetic construct
WIFPGDGSTKYNEKFKD

SEQ ID NO: 25 - skipped

SEQ ID NO: 26 - protein, 17 aa, synthetic construct
DINPYNGGIIYNQKFRG

SEQ ID NO: 27 - protein, 10 aa, synthetic construct
EVRRGSFFDY

SEQ ID NO: 28 - protein, 16 aa, synthetic construct
LIYWDDDKRYNPSLKS

SEQ ID NO: 29 - protein, 8 aa, synthetic construct
SPWDWFAY

SEQ ID NO: 30 - protein, 8 aa, synthetic construct
RAYGAMDY

SEQ ID NO: 31 - protein, 8 aa, synthetic construct
TGWDFFDI

SEQ ID NO: 32 - protein, 5 aa, synthetic construct
SYWIE

SEQ ID NO: 33 - protein, 17 aa, synthetic construct
EILPGSGITNYNEKFKG

SEQ ID NO: 34 - protein, 10 aa, synthetic construct
ETARARGFTY

SEQ ID NO: 35 - skipped

SEQ ID NO: 36 - protein, 11 aa, synthetic construct
KASQDVNTAVA

SEQ ID NO: 37 - protein, 7 aa, synthetic construct
SSSYRYT

SEQ ID NO: 38 - protein, 9 aa, synthetic construct
QQHYSTPWT

SEQ ID NO: 39 - protein, 11 aa, synthetic construct
KASQNVGTNVA

SEQ ID NO: 40 - protein, 7 aa, synthetic construct
SASYRYS

SEQ ID NO: 41 - protein, 9 aa, synthetic construct
QQYNSYPWT

SEQ ID NO: 42 - protein, 9 aa, synthetic construct
QQYNSYPYT

SEQ ID NO: 43 - protein, 11 aa, synthetic construct
KASEDIYHRLA

SEQ ID NO: 44 - protein, 7 aa, synthetic construct
GATSLET

SEQ ID NO: 45 - protein, 9 aa, synthetic construct
QQYWSPPFT

SEQ ID NO: 46 - protein, 11 aa, synthetic construct
RPSESIYSNLA

SEQ ID NO: 47 - protein, 7 aa, synthetic construct
AATNLAD

SEQ ID NO: 48 - protein, 9 aa, synthetic construct
QHFWGIPWT

SEQ ID NO: 49 - protein, 11 aa, synthetic construct
RASENIYSNLA

SEQ ID NO: 50 - protein, 7 aa, synthetic construct
AATNLGD

SEQ ID NO: 51 - protein, 9 aa, synthetic construct
QHFWGTPWT

SEQ ID NO: 52 - protein, 16 aa, synthetic construct
RSSKSLLHSNGITYLY

SEQ ID NO: 53 - protein, 7 aa, synthetic construct
QMSNLVS

SEQ ID NO: 54 - protein, 9 aa, synthetic construct
AQNLELPPT

SEQ ID NO: 55 - protein, 11 aa, synthetic construct
RASQDISNYLN

SEQ ID NO: 56 - protein, 7 aa, synthetic construct
SASNLHS

SEQ ID NO: 57 - protein, 9 aa, synthetic construct
QQYNMFPWT

SEQ ID NO: 58 - protein, 11 aa, synthetic construct
KASQDINSYLS

SEQ ID NO: 59 - protein, 7 aa, synthetic construct
RANKLVD

SEQ ID NO: 60 - protein, 9 aa, synthetic construct
LQYDEFPYT

SEQ ID NO: 61 - protein, 7 aa, synthetic construct
AATDLAD

SEQ ID NO: 62 - protein, 8 aa, synthetic construct
QLFWGTPT

SEQ ID NO: 63 - protein, 12 aa, synthetic construct
SVSSSISSSNLH

SEQ ID NO: 64 - protein, 7 aa, synthetic construct
GTSNLAS

SEQ ID NO: 65 - protein, 9 aa, synthetic construct
QQWSSYPLT

SEQ ID NO: 66 - protein, 11 aa, synthetic construct
KASQNVGTNIA

SEQ ID NO: 67 - protein, 9 aa, synthetic construct
QQYNTYPHT

SEQ ID NO: 68 - protein, 11 aa, synthetic construct
KASQNVGSNVA

SEQ ID NO: 69 - protein, 9 aa, synthetic construct
QQYKSYPLT

SEQ ID NO: 70 - protein, 11 aa, synthetic construct
ITSIDIDDDIN

SEQ ID NO: 71 - protein, 7 aa, synthetic construct
EGNTLRP

SEQ ID NO: 72 - protein, 9 aa, synthetic construct
LQSDNLPLT

SEQ ID NO: 73 - protein, 16 aa, synthetic construct
KSSKSLLHSEGITYLY

SEQ ID NO: 74 - protein, 17 aa, synthetic construct
DLNPYNAGIIYNQKFKG

SEQ ID NO: 75 - protein, 17 aa, synthetic construct
DLNPYNQGIIYNQKFKG

SEQ ID NO: 76 - protein, 17 aa, synthetic construct
DLNPYEGGIIYNQKFKG

SEQ ID NO: 77 - protein, 16 aa, synthetic construct
RSSKSLLHSNAITYLY

SEQ ID NO: 78 - protein, 16 aa, synthetic construct
RSSKSLLHSNQITYLY

SEQ ID NO: 79 - protein, 16 aa, synthetic construct
RSSKSLLHSEGITYLY

SEQ ID NO: 80 - protein, 9 aa, synthetic construct
QQYNAYPWT

SEQ ID NO: 81 - protein, 9 aa, synthetic construct
QQYESYPWT

SEQ ID NO: 82 - protein, 9 aa, synthetic construct
QQYNQYPWT

SEQ ID NO: 83 - protein, 118 aa, synthetic construct
QVTLKESGPGILQPSQTLSLTCSFSGFSLSTYGIGVGWIRQPSGKGLEWLAHIWWNNNKYFNTALKSRLTISKDTSNNQVFLKIASVDTADSATYYCARMGYDIMDYWGQGTSVTVSS

SEQ ID NO: 84 - protein, 118 aa, synthetic construct
QVTLKESGPGILQPSQTLSLTCSFSGFSLTISGMGVSWIRQPSGKGLEWLAHIYWDDDKRYNPSLKSRLTISKDTSSNQVFLEITSVDTADTATYYCVRAGWDFFDYWGQGTTLTVSS

SEQ ID NO: 85 - protein, 118 aa, synthetic construct
QVTLKESGPGILQPSQTLSLTCSFSGFSLSTSGMGVSWIRQPSGKGLEWLAHIYWDDDKRYNPSLKSRLTISKDTSSNRVFLKITSVDTADTATYYCARTGWDFFDYWGQGTTLTVSS

SEQ ID NO: 86 - protein, 119 aa, synthetic construct
EVLLQQSGPELVKPGASVKIACKASGYTLTDYNLNWVKQSHGKSLEWIGDLNPYNGGIIYNQKFKGKATLTVDKSSSTAYMELRSLTSEDIAVYYCAREGRGGAWFDSWGQGTLVTVSA

SEQ ID NO: 87 - protein, 119 aa, synthetic construct
EVQLRQSGPELVKPGTSMKISCKASAYSFTDYNMNWVKQSHGKNLEWIGLINPYNGGTRYNQNFKGKATITVDRSSTTAYMELLSLTSEDSAIYYCAREVRLGNALDYWGQGTSVTVSS

SEQ ID NO: 88 - protein, 119 aa, synthetic construct
EVQLQQSGPELVKPGASLKISCKASGYSFTGYNMNWVKQSHGKNLEWIGLINPSNGGSSYSQKFKGKATLTVDKSSSTAYMELLSLTSKDSAVYYCAREVRLGNALDYWGQGTSVTVSS

SEQ ID NO: 89 - protein, 118 aa, synthetic construct
QVTLKESGPGILQPSQTLSLTCSFSGFSLSTYGIGVGWIRQPSGKGLEWLAHIWWNDNKYYNTALKSRLTISKDTSNNQVFLKIASVDTADTATYYCARLAYDYVDSWGQGTTLTVSS

SEQ ID NO: 90 - protein, 119 aa, synthetic construct
EVQLQQSGPELVKPGASMKISCKASGYSFTGYNMNWVKQSQGKNLEWIGLINPYNGGTIYNQKFKGKATLTVDKSSTTAYMELLSLTSEDSAVYYCAREVRLGNAMDYWGQGTSVTVSS

SEQ ID NO: 91 - protein, 118 aa, synthetic construct
QGTLKESGPGILQPSQTLSLTCSFSGFSLSISGMGVSWIRQPSGKGLEWLAHIYWDDDKRYKPSLKSRLTISKDTSRNQVFLKITSVDTADTATYYCARSAYGMTDYWGQGTTLTVSS

SEQ ID NO: 92 - protein, 112 aa, synthetic construct
QVQLQQSGAELVKPGASVKLSCKASGYTFTNYDINWVRQRPEQGLEWIGWIFPGDGSTKYNEKFKDKATLTTDTSSSTAYMQLIRLTSEDSAVYFCARILYWGQGTTLTVSS

SEQ ID NO: 93 - protein, 119 aa, synthetic construct
EVLLQQSGPELVKPGASVKITCKASGYTFTDYNMNWVKQSHGKSLEWIGDINPYNGGIIYNQKFRGKATLTIDKSSSTAYMELRSLTSEDTAVYYCAREVRRGSFFDYWGQGTTLTVSS

SEQ ID NO: 94 - protein, 118 aa, synthetic construct
QVTLKESGPGILQPSQTLSLTCSFSGFSLSTSGMGVSWIRQPSGKGLEWLALIYWDDDKRYNPSLKSRLTISKDASSNQVFLKITSVDTADTATYYCIQSPWDWFAYWGQGTLVTVSA

SEQ ID NO: 95 - protein, 118 aa, synthetic construct
QVTLKESGPGILQPSQTLSLTCSFSGFSLSTSGMGVSWIRQPSGKGLEWLAHIYWDDDKRYNPSLKSRLTISKDTSRNQVFLKITSVDTADTATYYCARRAYGAMDYWGHGTSVTVSS

SEQ ID NO: 96 - protein, 118 aa, synthetic construct
QVTLKESGPGILQPSQTLSLTCSFSGFSLNTSGMGVSWIRQPSGKGLEWLAHIYWDDDKRYNPSLKSRLTISKDTSRNQVFLKITGVDTADTAAYYCARTGWDFFDIWGQGTTLTVSS

SEQ ID NO: 97 - protein, 119 aa, synthetic construct
QVQLQQSGAELMKPGASVKISCKATGYTFSSYWIEWVKQRPGHGLEWIGEILPGSGITNYNEKFKGKATFTADTSSNTAYMQLSSLTSEDSAVYYCARETARARGFTYWGQGTLVTVSA

SEQ ID NO: 98 - protein, 119 aa, synthetic construct
EVLLQQSGPELVKPGASVKIACKASGYTLTDYNLNWVKQSHGKSLEWIGDLNPYNAGIIYNQKFKGKATLTVDKSSSTAYMELRSLTSEDIAVYYCAREGRGGAWFDSWGQGTLVTVSA

SEQ ID NO: 99 - protein, 119 aa, synthetic construct
EVLLQQSGPELVKPGASVKIACKASGYTLTDYNLNWVKQSHGKSLEWIGDLNPYNQGIIYNQKFKGKATLTVDKSSSTAYMELRSLTSEDIAVYYCAREGRGGAWFDSWGQGTLVTVSA

SEQ ID NO: 100 - protein, 119 aa, synthetic construct
EVLLQQSGPELVKPGASVKIACKASGYTLTDYNLNWVKQSHGKSLEWIGDLNPYEGGIIYNQKFKGKATLTVDKSSSTAYMELRSLTSEDIAVYYCAREGRGGAWFDSWGQGTLVTVSA

SEQ ID NO: 101 - skipped

SEQ ID NO: 102 - protein, 107 aa, synthetic construct
DIVMTQSHKFMSTSVGDRVSITCKASQDVNTAVAWYQQKPGQSPKFLIYSSSYRYTGVPDRFTGSGSGTDFTFTISSVQAEDLAVYYCQQHYSTPWTFGGGTKLEIK

SEQ ID NO: 103 - protein, 107 aa, synthetic construct
DIVMTQSQKFMSTSVGDRVSVTCKASQNVGTNVAWYQQKPGQSPKGLIYSASYRYSGVPDRFTGSGSGTDFTLTISNVQSEDLAEYFCQQYNSYPWTFGGGTKLEIK

SEQ ID NO: 104 - protein, 107 aa, synthetic construct
DIVMTQSQKFMSTSVGDRVSVTCKASQNVGTNVAWYQQKPGQSPKGLIYSASYRYSGVPDRFTGSGSGTDFTLTINNVQSEDLAEYFCQQYNSYPYTFGGGTKLEIK

SEQ ID NO: 105 - protein, 107 aa, synthetic construct
DIQMTQSSSSFSVSLGDRVTITCKASEDIYHRLAWYQQKPGNAPRLLISGATSLETGIPSRFSGSGSGKDYALSITSLQTEDVGTYYCQQYWSPPFTFGSGTKLEIK

SEQ ID NO: 106 - protein, 107 aa, synthetic construct
DIQMTQSPASLSVSVGETVTITCRPSESIYSNLAWYQQKQGKSPQLLVYAATNLADGVPSRFSGSGSGTQYSLKINSLQSEDFGTYYCQHFWGIPWTFGGGTKLEIK

SEQ ID NO: 107 - protein, 107 aa, synthetic construct
DIQMTQSPASLSVSVGETVTITCRASENIYSNLAWYQQKQGKSPQLLVYAATNLGDGAPSRFSGSGSGTQYSLKINSLQSEDFGSYYCQHFWGTPWTFGGGTKLEIK

SEQ ID NO: 108 - protein, 112 aa, synthetic construct
DIVMTQAAFSNPVTLGTSASISCRSSKSLLHSNGITYLYWYLQKPGQSPQLLIYQMSNLVSGVPDRFSSSGSGTDFTLRISRVEAEDVGVYYCAQNLELPPTFGAGTKLELK

SEQ ID NO: 109 - protein, 107 aa, synthetic construct
DIQMTQSPASLSVSVGETVTITCRASENIYSNLAWYQQKQGKSPQLLVSAATNLADGVPSRFSGSGSGTQYSLKIISLQSVDFGSYYCQHFWGTPWTFGGGTKLEIK

SEQ ID NO: 110 - protein, 107 aa, synthetic construct
DIQMTQTTSSLSASLGDRVTISCRASQDISNYLNWYQQKPDGTVKLLIHSASNLHSGVPSRFSGSGSGTDYSLTISNLEQEDIATYFCQQYNMFPWTFGGGTKLEIK

SEQ ID NO: 111 - protein, 107 aa, synthetic construct
DNKMTQSPSSMYASLGERVTITCKASQDINSYLSWFQQKPGKSPKTLIYRANKLVDGVPSRFSGSGSGQDYSLTISSLEYEDMGIYHCLQYDEFPYTFGGGTKLEIK

SEQ ID NO: 112 - protein, 106 aa, synthetic construct
DIQMTQSPASLSVSVGETVTITCRASENIYSNLAWYQQKQGKSPQLLVYAATDLADGVPSRFSGSGSGTQYSLKINSLQSEDFGNYHCQLFWGTPTFGGGTKLEIK

SEQ ID NO: 113 - protein, 108 aa, synthetic construct
EIVLTQSPALMAASPGEKVTITCSVSSSISSSNLHWYQQKSETSPKPWIYGTSNLASGVPVRFSGSGSGTSYSLTISSMEAEDAATYYCQQWSSYPLTFGAGTKLELK

SEQ ID NO: 114 - protein, 107 aa, synthetic construct
DIVMTQSQKFMSTSVGDRVSVTCKASQNVGTNIAWFQQKPGQSPEALIYSASYRYSGVPDRFTGSGSGTDFTLTISNVQSEDLAEYFCQQYNTYPHTFGGGTKLEIR

SEQ ID NO: 115 - protein, 107 aa, synthetic construct
DIVMTQSQKFMSTSVGDRVSVTCKASQNVGSNVAWYQQKPGQSPKALIYSASYRYSGVPDRFTGSGSGTDFTLTITNVQSEDLAEYFCQQYKSYPLTFGAGTKLELK

SEQ ID NO: 116 - protein, 107 aa, synthetic construct
ETTVTQSPASLSMAIGEKVTIRCITSIDIDDDINWYQQKPGEPPNLLISEGNTLRPGVPSRFSSSGYGTDFVFTIENMLSEDVADYYCLQSDNLPLTFGGGTKLEIK

SEQ ID NO: 117 - protein, 112 aa, synthetic construct
DIVMTQAAFSNPVTLGTSASISCRSSKSLLHSNAITYLYWYLQKPGQSPQLLIYQMSNLVSGVPDRFSSSGSGTDFTLRISRVEAEDVGVYYCAQNLELPPTFGAGTKLELK

SEQ ID NO: 118 - protein, 112 aa, synthetic construct
DIVMTQAAFSNPVTLGTSASISCRSSKSLLHSNQITYLYWYLQKPGQSPQLLIYQMSNLVSGVPDRFSSSGSGTDFTLRISRVEAEDVGVYYCAQNLELPPTFGAGTKLELK

SEQ ID NO: 119 - protein, 112 aa, synthetic construct
DIVMTQAAFSNPVTLGTSASISCRSSKSLLHSEGITYLYWYLQKPGQSPQLLIYQMSNLVSGVPDRFSSSGSGTDFTLRISRVEAEDVGVYYCAQNLELPPTFGAGTKLELK

SEQ ID NO: 120 - protein, 107 aa, synthetic construct
DIVMTQSQKFMSTSVGDRVSVTCKASQNVGTNVAWYQQKPGQSPKGLIYSASYRYSGVPDRFTGSGSGTDFTLTISNVQSEDLAEYFCQQYNAYPWTFGGGTKLEIK

SEQ ID NO: 121 - protein, 107 aa, synthetic construct
DIVMTQSQKFMSTSVGDRVSVTCKASQNVGTNVAWYQQKPGQSPKGLIYSASYRYSGVPDRFTGSGSGTDFTLTISNVQSEDLAEYFCQQYESYPWTFGGGTKLEIK

SEQ ID NO: 122 - protein, 107 aa, synthetic construct
DIVMTQSQKFMSTSVGDRVSVTCKASQNVGTNVAWYQQKPGQSPKGLIYSASYRYSGVPDRFTGSGSGTDFTLTISNVQSEDLAEYFCQQYNQYPWTFGGGTKLEIK

SEQ ID NO: 123 - skipped

SEQ ID NO: 124 - protein, 118 aa, synthetic construct
QVQLQESGPGLVKPSETLSLTCTFSGFSLSTYGIGVGWIRQPPGKGLEWIAHIWWNNNKYFNTALKSRLTISKDTSKNQVSLKLSSVTAADTAVYYCARMGYDIMDYWGQGTLVTVSS

SEQ ID NO: 125 - protein, 118 aa, synthetic construct
QVTLQESGPGLVKPSETLSLTCSFSGFSLSTYGIGVGWIRQPPGKGLEWLAHIWWNNNKYFNTALKSRLTISKDTSKNQVSLKLSSVTAADTATYYCARMGYDIMDYWGQGTSVTVSS

SEQ ID NO: 126 - protein, 118 aa, synthetic construct
EVQLLESGGGLVQPGGSLRLSCAFSGFSLSTYGIGVGWIRQAPGKGLEWVAHIWWNNNKYFNTALKSRLTISKDTSKNTVYLQMNSLRAEDTAVYYCAKMGYDIMDYWGQGTTVTVSS

SEQ ID NO: 127 - protein, 118 aa, synthetic construct
QVTLLESGGGLVQPGGSLRLSCSFSGFSLSTYGIGVGWIRQAPGKGLEWLAHIWWNNNKYFNTALKSRLTISKDTSKNTVYLQMNSVRAEDTAVYYCARMGYDIMDYWGQGTTVTVSS

SEQ ID NO: 128 - protein, 107 aa, synthetic construct
DIQMTQSPSSLSTSVGDRVTITCKASQDVNTAVAWYQQKPGKAPKFLIYSSSYRYTGVPDRFSGSGSGTDFTFTISSLQPEDFAVYYCQQHYSTPWTFGQGTKVEIK

SEQ ID NO: 129 - protein, 107 aa, synthetic construct
DIVMTQSPSSLSTSVGDRVTITCKASQDVNTAVAWYQQKPGKSPKFLIYSSSYRYTGVPDRFSGSGSGTDFTFTISSVQPEDFAVYYCQQHYSTPWTFGGGTKVEIK

SEQ ID NO: 130 - protein, 107 aa, synthetic construct
DIVMTQSPATLSTSPGERATLSCKASQDVNTAVAWYQQKPGQAPRFLIYSSSYRYTGVPARFSGSGSGTEFTFTISSLQSEDFAVYYCQQHYSTPWTFGGGTKVEIK

SEQ ID NO: 131 - protein, 107 aa, synthetic construct
DIVMTQSPATLSTSPGERVTISCKASQDVNTAVAWYQQKPGQSPRFLIYSSSYRYTGVPDRFSGSGSGTDFTFTISSVQSEDFAVYYCQQHYSTPWTFGGGTKVEIK

SEQ ID NO: 132 - protein, 119 aa, synthetic construct
EVQLVQSGAEVKKPGASVKVSCKASGYTFTDYNLNWVRQATGQGLEWMGDLNPYNQGIIYNQKFKGRVTMTVDTSISTAYMELSSLRSEDTAVYYCAREGRGGAWFDSWGQGTLVTVSS

SEQ ID NO: 133 - protein, 119 aa, synthetic construct
EVQLVQSGAEVKKPGASVKVSCKASGYTFTDYNLNWVRQATGQGLEWMGDLNPYNQGIIYNQKFKGRVTLTVDKSISTAYMELSSLRSEDTAVYYCAREGRGGAWFDSWGQGTLVTVSS

SEQ ID NO: 134 - protein, 119 aa, synthetic construct
EVQLVQSGAEVKKPGASVKVSCKASGYTFTDYNLNWVRQATGQGLEWIGDLNPYNQGIIYNQKFKGRATLTVDKSISTAYMELSSLRSEDTAVYYCAREGRGGAWFDSWGQGTLVTVSS

SEQ ID NO: 135 - protein, 119 aa, synthetic construct
EVQLVQSGAEVKKPGASVKVSCKASGYTLTDYNLNWVRQATGQGLEWIGDLNPYNQGIIYNQKFKGRATLTVNKSISTAYMELSSLRSEDTAVYYCAREGRGGAWFDSWGQGTLVTVSS

SEQ ID NO: 136 - protein, 107 aa, synthetic construct
DIQMTQSPSSLSASVGDRVTITCKASEDIYHRLAWYQQKPGKAPKLLIYGATSLETGVPSRFSGSGSGTDFTFTISSLQPEDIATYYCQQYWSPPFTFGGGTKVEIK

SEQ ID NO: 137 - protein, 107 aa, synthetic construct
DIQMTQSPSSLSASVGDRVTITCKASEDIYHRLAWYQQKPGKAPKLLIYGATSLETGVPSRFSGSGSGTDYTFTISSLQPEDIATYYCQQYWSPPFTFGGGTKVEIK

SEQ ID NO: 138 - protein, 107 aa, synthetic construct
DIQMTQSPSSLSASVGDRVTITCKASEDIYHRLAWYQQKPGKAPKLLISGATSLETGVPSRFSGSGSGTDYTFTISSLQPEDIATYYCQQYWSPPFTFGGGTKVEIK

SEQ ID NO: 139 - protein, 107 aa, synthetic construct
DIQMTQSPSSLSASVGDRVTITCKASEDIYHRLAWYQQKPGKAPKLLISGATSLETGIPSRFSGSGSGTDYTFTISSLQPEDIATYYCQQYWSPPFTFGGGTKVEIK

SEQ ID NO: 140 - protein, 118 aa, synthetic construct
QVTLKESGPALVKPTQTLTLTCTFSGFSLSTYGIGVGWIRQPPGKALEWLAHIWWNDNKYYNTALKSRLTISKDTSKNQVVLTMTNMDPVDTATYYCARLAYDYVDSWGQGTTLTVSS

SEQ ID NO: 141 - protein, 118 aa, synthetic construct
QVTLKESGPALVKPTQTLTLTCTFSGFSLSTYGIGVGWIRQPPGKGLEWLAHIWWNDNKYYNTALKSRLTISKDTSKNQVVLTMTNMDPVDTATYYCARLAYDYVDSWGQGTTLTVSS

SEQ ID NO: 142 - protein, 112 aa, synthetic construct
DIVMTQTPLSLSVTPGQPASISCRSSKSLLHSEGITYLYWYLQKPGQSPQLLIYQMSNLVSGVPDRFSGSGSGTDFTLKISRVEAEDVGVYYCAQNLELPPTFGQGTKLEIK

SEQ ID NO: 143 - protein, 112 aa, synthetic construct
DIVMTQTPLSLSVTPGQPASISCRSSKSLLHSEGITYLYWYLQKPGQSPQLLIYQMSNLVSGVPDRFSSSGSGTDFTLKISRVEAEDVGVYYCAQNLELPPTFGQGTKLEIK

SEQ ID NO: 144 - protein, 118 aa, synthetic construct
QITLKESGPTLVKPTQTLTLTCTFSGFSLSTYGIGVGWIRQPPGKALEWLAHIWWNDNKYYNTALKSRLTITKDTSKNQVVLTMTNMDPVDTATYYCARLAYDYVDSWGQGTLVTVSS

SEQ ID NO: 145 - protein, 118 aa, synthetic construct
QITLKESGPALVKPTQTLTLTCTFSGFSLSTYGIGVGWIRQPPGKALEWLAHIWWNDNKYYNTALKSRLTITKDTSKNQVFLTMTNMDPVDTATYYCARLAYDYVDSWGQGTLVTVSS

SEQ ID NO: 146 - protein, 112 aa, synthetic construct
DIVMTQTPLSLSVTPGQPASISCKSSKSLLHSEGITYLYWYLQKPGQSPQLLIYQMSNLVSGVPDRFSGSGSGTDFTLKISRVEAEDVGVYYCAQNLELPPTFGQGTKLEIK

SEQ ID NO: 147 - protein, 112 aa, synthetic construct
DIVMTQSPLSLSVTPGEPASISCRSSKSLLHSEGITYLYWYLQKPGQSPQLLIYQMSNLVSGVPDRFSGSGSGTDFTLKISRVEAEDVGVYYCAQNLELPPTFGQGTKLEIK

SEQ ID NO: 148 - protein, 329 aa, synthetic construct
ASTKGPSVFPLAPSSKSTSGGTAALGCLVKDYFPEPVTVSWNSGALTSGVHTFPAVLQSSGLYSLSSVVTVPSSSLGTQTYICNVNHKPSNTKVDKKVEPKSCDKTHTCPPCPAPEAAGAPSVFLFPPKPKDTLMISRTPEVTCVVVDVSHEDPEVKFNWYVDGVEVHNAKTKPREEQYNSTYRVVSVLTVLHQDWLNGKEYKCKVSNKALPAPIEKTISKAKGQPREPQVYTLPPSREEMTKNQVSLTCLVKGFYPSDIAVEWESNGQPENNYKTTPPVLDSDGSFFLYSKLTVDKSRWQQGNVFSCSVMHEALHNHYTQKSLSLSPG

SEQ ID NO: 149 - protein, 107 aa, synthetic construct [sequence omitted]

SEQ ID NO: 150 - protein, 447 aa, synthetic construct
QVTLKESGPGILQPSQTLSLTCSFSGFSLSTYGIGVGWIRQPSGKGLEWLAHIWWNNNKYFNTALKSRLTISKDTSNNQVFLKIASVDTADSATYYCARMGYDIMDYWGQGTSVTVSSASTKGPSVFPLAPSSKSTSGGTAALGCLVKDYFPEPVTVSWNSGALTSGVHTFPAVLQSSGLYSLSSVVTVPSSSLGTQTYICNVNHKPSNTKVDKKVEPKSCDKTHTCPPCPAPEAAGAPSVFLFPPKPKDTLMISRTPEVTCVVVDVSHEDPEVKFNWYVDGVEVHNAKTKPREEQYNSTYRVVSVLTVLHQDWLNGKEYKCKVSNKALPAPIEKTISKAKGQPREPQVYTLPPSREEMTKNQVSLTCLVKGFYPSDIAVEWESNGQPENNYKTTPPVLDSDGSFFLYSKLTVDKSRWQQGNVFSCSVMHEALHNHYTQKSLSLSPG

SEQ ID NO: 151 - protein, 447 aa, synthetic construct
QVTLKESGPGILQPSQTLSLTCSFSGFSLTISGMGVSWIRQPSGKGLEWLAHIYWDDDKRYNPSLKSRLTISKDTSSNQVFLEITSVDTADTATYYCVRAGWDFFDYWGQGTTLTVSSASTKGPSVFPLAPSSKSTSGGTAALGCLVKDYFPEPVTVSWNSGALTSGVHTFPAVLQSSGLYSLSSVVTVPSSSLGTQTYICNVNHKPSNTKVDKKVEPKSCDKTHTCPPCPAPEAAGAPSVFLFPPKPKDTLMISRTPEVTCVVVDVSHEDPEVKFNWYVDGVEVHNAKTKPREEQYNSTYRVVSVLTVLHQDWLNGKEYKCKVSNKALPAPIEKTISKAKGQPREPQVYTLPPSREEMTKNQVSLTCLVKGFYPSDIAVEWESNGQPENNYKTTPPVLDSDGSFFLYSKLTVDKSRWQQGNVFSCSVMHEALHNHYTQKSLSLSPG

SEQ ID NO: 152 - protein, 447 aa, synthetic construct
QVTLKESGPGILQPSQTLSLTCSFSGFSLSTSGMGVSWIRQPSGKGLEWLAHIYWDDDKRYNPSLKSRLTISKDTSSNRVFLKITSVDTADTATYYCARTGWDFFDYWGQGTTLTVSSASTKGPSVFPLAPSSKSTSGGTAALGCLVKDYFPEPVTVSWNSGALTSGVHTFPAVLQSSGLYSLSSVVTVPSSSLGTQTYICNVNHKPSNTKVDKKVEPKSCDKTHTCPPCPAPEAAGAPSVFLFPPKPKDTLMISRTPEVTCVVVDVSHEDPEVKFNWYVDGVEVHNAKTKPREEQYNSTYRVVSVLTVLHQDWLNGKEYKCKVSNKALPAPIEKTISKAKGQPREPQVYTLPPSREEMTKNQVSLTCLVKGFYPSDIAVEWESNGQPENNYKTTPPVLDSDGSFFLYSKLTVDKSRWQQGNVFSCSVMHEALHNHYTQKSLSLSPG

SEQ ID NO: 153 - protein, 448 aa, synthetic construct
EVLLQQSGPELVKPGASVKIACKASGYTLTDYNLNWVKQSHGKSLEWIGDLNPYNGGIIYNQKFKGKATLTVDKSSSTAYMELRSLTSEDIAVYYCAREGRGGAWFDSWGQGTLVTVSAASTKGPSVFPLAPSSKSTSGGTAALGCLVKDYFPEPVTVSWNSGALTSGVHTFPAVLQSSGLYSLSSVVTVPSSSLGTQTYICNVNHKPSNTKVDKKVEPKSCDKTHTCPPCPAPEAAGAPSVFLFPPKPKDTLMISRTPEVTCVVVDVSHEDPEVKFNWYVDGVEVHNAKTKPREEQYNSTYRVVSVLTVLHQDWLNGKEYKCKVSNKALPAPIEKTISKAKGQPREPQVYTLPPSREEMTKNQVSLTCLVKGFYPSDIAVEWESNGQPENNYKTTPPVLDSDGSFFLYSKLTVDKSRWQQGNVFSCSVMHEALHNHYTQKSLSLSPG

SEQ ID NO: 154 - protein, 448 aa, synthetic construct
EVQLRQSGPELVKPGTSMKISCKASAYSFTDYNMNWVKQSHGKNLEWIGLINPYNGGTRYNQNFKGKATITVDRSSTTAYMELLSLTSEDSAIYYCAREVRLGNALDYWGQGTSVTVSSASTKGPSVFPLAPSSKSTSGGTAALGCLVKDYFPEPVTVSWNSGALTSGVHTFPAVLQSSGLYSLSSVVTVPSSSLGTQTYICNVNHKPSNTKVDKKVEPKSCDKTHTCPPCPAPEAAGAPSVFLFPPKPKDTLMISRTPEVTCVVVDVSHEDPEVKFNWYVDGVEVHNAKTKPREEQYNSTYRVVSVLTVLHQDWLNGKEYKCKVSNKALPAPIEKTISKAKGQPREPQVYTLPPSREEMTKNQVSLTCLVKGFYPSDIAVEWESNGQPENNYKTTPPVLDSDGSFFLYSKLTVDKSRWQQGNVFSCSVMHEALHNHYTQKSLSLSPG

SEQ ID NO: 155 - protein, 448 aa, synthetic construct
EVQLQQSGPELVKPGASLKISCKASGYSFTGYNMNWVKQSHGKNLEWIGLINPSNGGSSYSQKFKGKATLTVDKSSSTAYMELLSLTSKDSAVYYCAREVRLGNALDYWGQGTSVTVSSASTKGPSVFPLAPSSKSTSGGTAALGCLVKDYFPEPVTVSWNSGALTSGVHTFPAVLQSSGLYSLSSVVTVPSSSLGTQTYICNVNHKPSNTKVDKKVEPKSCDKTHTCPPCPAPEAAGAPSVFLFPPKPKDTLMISRTPEVTCVVVDVSHEDPEVKFNWYVDGVEVHNAKTKPREEQYNSTYRVVSVLTVLHQDWLNGKEYKCKVSNKALPAPIEKTISKAKGQPREPQVYTLPPSREEMTKNQVSLTCLVKGFYPSDIAVEWESNGQPENNYKTTPPVLDSDGSFFLYSKLTVDKSRWQQGNVFSCSVMHEALHNHYTQKSLSLSPG

SEQ ID NO: 156 - protein, 447 aa, synthetic construct
QVTLKESGPGILQPSQTLSLTCSFSGFSLSTYGIGVGWIRQPSGKGLEWLAHIWWNDNKYYNTALKSRLTISKDTSNNQVFLKIASVDTADTATYYCARLAYDYVDSWGQGTTLTVSSASTKGPSVFPLAPSSKSTSGGTAALGCLVKDYFPEPVTVSWNSGALTSGVHTFPAVLQSSGLYSLSSVVTVPSSSLGTQTYICNVNHKPSNTKVDKKVEPKSCDKTHTCPPCPAPEAAGAPSVFLFPPKPKDTLMISRTPEVTCVVVDVSHEDPEVKFNWYVDGVEVHNAKTKPREEQYNSTYRVVSVLTVLHQDWLNGKEYKCKVSNKALPAPIEKTISKAKGQPREPQVYTLPPSREEMTKNQVSLTCLVKGFYPSDIAVEWESNGQPENNYKTTPPVLDSDGSFFLYSKLTVDKSRWQQGNVFSCSVMHEALHNHYTQKSLSLSPG

SEQ ID NO: 157 - protein, 448 aa, synthetic construct
EVQLQQSGPELVKPGASMKISCKASGYSFTGYNMNWVKQSQGKNLEWIGLINPYNGGTIYNQKFKGKATLTVDKSSTTAYMELLSLTSEDSAVYYCAREVRLGNAMDYWGQGTSVTVSSASTKGPSVFPLAPSSKSTSGGTAALGCLVKDYFPEPVTVSWNSGALTSGVHTFPAVLQSSGLYSLSSVVTVPSSSLGTQTYICNVNHKPSNTKVDKKVEPKSCDKTHTCPPCPAPEAAGAPSVFLFPPKPKDTLMISRTPEVTCVVVDVSHEDPEVKFNWYVDGVEVHNAKTKPREEQYNSTYRVVSVLTVLHQDWLNGKEYKCKVSNKALPAPIEKTISKAKGQPREPQVYTLPPSREEMTKNQVSLTCLVKGFYPSDIAVEWESNGQPENNYKTTPPVLDSDGSFFLYSKLTVDKSRWQQGNVFSCSVMHEALHNHYTQKSLSLSPG

SEQ ID NO: 158 - protein, 447 aa, synthetic construct
QGTLKESGPGILQPSQTLSLTCSFSGFSLSISGMGVSWIRQPSGKGLEWLAHIYWDDDKRYKPSLKSRLTISKDTSRNQVFLKITSVDTADTATYYCARSAYGMTDYWGQGTTLTVSSASTKGPSVFPLAPSSKSTSGGTAALGCLVKDYFPEPVTVSWNSGALTSGVHTFPAVLQSSGLYSLSSVVTVPSSSLGTQTYICNVNHKPSNTKVDKKVEPKSCDKTHTCPPCPAPEAAGAPSVFLFPPKPKDTLMISRTPEVTCVVVDVSHEDPEVKFNWYVDGVEVHNAKTKPREEQYNSTYRVVSVLTVLHQDWLNGKEYKCKVSNKALPAPIEKTISKAKGQPREPQVYTLPPSREEMTKNQVSLTCLVKGFYPSDIAVEWESNGQPENNYKTTPPVLDSDGSFFLYSKLTVDKSRWQQGNVFSCSVMHEALHNHYTQKSLSLSPG

SEQ ID NO: 159 - protein, 441 aa, synthetic construct
QVQLQQSGAELVKPGASVKLSCKASGYTFTNYDINWVRQRPEQGLEWIGWIFPGDGSTKYNEKFKDKATLTTDTSSSTAYMQLIRLTSEDSAVYFCARILYWGQGTTLTVSSASTKGPSVFPLAPSSKSTSGGTAALGCLVKDYFPEPVTVSWNSGALTSGVHTFPAVLQSSGLYSLSSVVTVPSSSLGTQTYICNVNHKPSNTKVDKKVEPKSCDKTHTCPPCPAPEAAGAPSVFLFPPKPKDTLMISRTPEVTCVVVDVSHEDPEVKFNWYVDGVEVHNAKTKPREEQYNSTYRVVSVLTVLHQDWLNGKEYKCKVSNKALPAPIEKTISKAKGQPREPQVYTLPPSREEMTKNQVSLTCLVKGFYPSDIAVEWESNGQPENNYKTTPPVLDSDGSFFLYSKLTVDKSRWQQGNVFSCSVMHEALHNHYTQKSLSLSPG

SEQ ID NO: 160 - protein, 448 aa, synthetic construct
EVLLQQSGPELVKPGASVKITCKASGYTFTDYNMNWVKQSHGKSLEWIGDINPYNGGIIYNQKFRGKATLTIDKSSSTAYMELRSLTSEDTAVYYCAREVRRGSFFDYWGQGTTLTVSSASTKGPSVFPLAPSSKSTSGGTAALGCLVKDYFPEPVTVSWNSGALTSGVHTFPAVLQSSGLYSLSSVVTVPSSSLGTQTYICNVNHKPSNTKVDKKVEPKSCDKTHTCPPCPAPEAAGAPSVFLFPPKPKDTLMISRTPEVTCVVVDVSHEDPEVKFNWYVDGVEVHNAKTKPREEQYNSTYRVVSVLTVLHQDWLNGKEYKCKVSNKALPAPIEKTISKAKGQPREPQVYTLPPSREEMTKNQVSLTCLVKGFYPSDIAVEWESNGQPENNYKTTPPVLDSDGSFFLYSKLTVDKSRWQQGNVFSCSVMHEALHNHYTQKSLSLSPG

SEQ ID NO: 161 - protein, 447 aa, synthetic construct
QVTLKESGPGILQPSQTLSLTCSFSGFSLSTSGMGVSWIRQPSGKGLEWLALIYWDDDKRYNPSLKSRLTISKDASSNQVFLKITSVDTADTATYYCIQSPWDWFAYWGQGTLVTVSAASTKGPSVFPLAPSSKSTSGGTAALGCLVKDYFPEPVTVSWNSGALTSGVHTFPAVLQSSGLYSLSSVVTVPSSSLGTQTYICNVNHKPSNTKVDKKVEPKSCDKTHTCPPCPAPEAAGAPSVFLFPPKPKDTLMISRTPEVTCVVVDVSHEDPEVKFNWYVDGVEVHNAKTKPREEQYNSTYRVVSVLTVLHQDWLNGKEYKCKVSNKALPAPIEKTISKAKGQPREPQVYTLPPSREEMTKNQVSLTCLVKGFYPSDIAVEWESNGQPENNYKTTPPVLDSDGSFFLYSKLTVDKSRWQQGNVFSCSVMHEALHNHYTQKSLSLSPG

SEQ ID NO: 162 - protein, 447 aa, synthetic construct
QVTLKESGPGILQPSQTLSLTCSFSGFSLSTSGMGVSWIRQPSGKGLEWLAHIYWDDDKRYNPSLKSRLTISKDTSRNQVFLKITSVDTADTATYYCARRAYGAMDYWGHGTSVTVSSASTKGPSVFPLAPSSKSTSGGTAALGCLVKDYFPEPVTVSWNSGALTSGVHTFPAVLQSSGLYSLSSVVTVPSSSLGTQTYICNVNHKPSNTKVDKKVEPKSCDKTHTCPPCPAPEAAGAPSVFLFPPKPKDTLMISRTPEVTCVVVDVSHEDPEVKFNWYVDGVEVHNAKTKPREEQYNSTYRVVSVLTVLHQDWLNGKEYKCKVSNKALPAPIEKTISKAKGQPREPQVYTLPPSREEMTKNQVSLTCLVKGFYPSDIAVEWESNGQPENNYKTTPPVLDSDGSFFLYSKLTVDKSRWQQGNVFSCSVMHEALHNHYTQKSLSLSPG

SEQ ID NO: 163 - protein, 447 aa, synthetic construct
QVTLKESGPGILQPSQTLSLTCSFSGFSLNTSGMGVSWIRQPSGKGLEWLAHIYWDDDKRYNPSLKSRLTISKDTSRNQVFLKITGVDTADTAAYYCARTGWDFFDIWGQGTTLTVSSASTKGPSVFPLAPSSKSTSGGTAALGCLVKDYFPEPVTVSWNSGALTSGVHTFPAVLQSSGLYSLSSVVTVPSSSLGTQTYICNVNHKPSNTKVDKKVEPKSCDKTHTCPPCPAPEAAGAPSVFLFPPKPKDTLMISRTPEVTCVVVDVSHEDPEVKFNWYVDGVEVHNAKTKPREEQYNSTYRVVSVLTVLHQDWLNGKEYKCKVSNKALPAPIEKTISKAKGQPREPQVYTLPPSREEMTKNQVSLTCLVKGFYPSDIAVEWESNGQPENNYKTTPPVLDSDGSFFLYSKLTVDKSRWQQGNVFSCSVMHEALHNHYTQKSLSLSPG

SEQ ID NO: 164 - protein, 448 aa, synthetic construct
QVQLQQSGAELMKPGASVKISCKATGYTFSSYWIEWVKQRPGHGLEWIGEILPGSGITNYNEKFKGKATFTADTSSNTAYMQLSSLTSEDSAVYYCARETARARGFTYWGQGTLVTVSAASTKGPSVFPLAPSSKSTSGGTAALGCLVKDYFPEPVTVSWNSGALTSGVHTFPAVLQSSGLYSLSSVVTVPSSSLGTQTYICNVNHKPSNTKVDKKVEPKSCDKTHTCPPCPAPEAAGAPSVFLFPPKPKDTLMISRTPEVTCVVVDVSHEDPEVKFNWYVDGVEVHNAKTKPREEQYNSTYRVVSVLTVLHQDWLNGKEYKCKVSNKALPAPIEKTISKAKGQPREPQVYTLPPSREEMTKNQVSLTCLVKGFYPSDIAVEWESNGQPENNYKTTPPVLDSDGSFFLYSKLTVDKSRWQQGNVFSCSVMHEALHNHYTQKSLSLSPG

SEQ ID NO: 165 - skipped

SEQ ID NO: 166 - protein, 448 aa, synthetic construct
EVLLQQSGPELVKPGASVKIACKASGYTLTDYNLNWVKQSHGKSLEWIGDLNPYNAGIIYNQKFKGKATLTVDKSSSTAYMELRSLTSEDIAVYYCAREGRGGAWFDSWGQGTLVTVSAASTKGPSVFPLAPSSKSTSGGTAALGCLVKDYFPEPVTVSWNSGALTSGVHTFPAVLQSSGLYSLSSVVTVPSSSLGTQTYICNVNHKPSNTKVDKKVEPKSCDKTHTCPPCPAPEAAGAPSVFLFPPKPKDTLMISRTPEVTCVVVDVSHEDPEVKFNWYVDGVEVHNAKTKPREEQYNSTYRVVSVLTVLHQDWLNGKEYKCKVSNKALPAPIEKTISKAKGQPREPQVYTLPPSREEMTKNQVSLTCLVKGFYPSDIAVEWESNGQPENNYKTTPPVLDSDGSFFLYSKLTVDKSRWQQGNVFSCSVMHEALHNHYTQKSLSLSPG

SEQ ID NO: 167 - protein, 448 aa, synthetic construct
EVLLQQSGPELVKPGASVKIACKASGYTLTDYNLNWVKQSHGKSLEWIGDLNPYNQGIIYNQKFKGKATLTVDKSSSTAYMELRSLTSEDIAVYYCAREGRGGAWFDSWGQGTLVTVSAASTKGPSVFPLAPSSKSTSGGTAALGCLVKDYFPEPVTVSWNSGALTSGVHTFPAVLQSSGLYSLSSVVTVPSSSLGTQTYICNVNHKPSNTKVDKKVEPKSCDKTHTCPPCPAPEAAGAPSVFLFPPKPKDTLMISRTPEVTCVVVDVSHEDPEVKFNWYVDGVEVHNAKTKPREEQYNSTYRVVSVLTVLHQDWLNGKEYKCKVSNKALPAPIEKTISKAKGQPREPQVYTLPPSREEMTKNQVSLTCLVKGFYPSDIAVEWESNGQPENNYKTTPPVLDSDGSFFLYSKLTVDKSRWQQGNVFSCSVMHEALHNHYTQKSLSLSPG

SEQ ID NO: 168 - protein, 448 aa, synthetic construct
EVLLQQSGPELVKPGASVKIACKASGYTLTDYNLNWVKQSHGKSLEWIGDLNPYEGGIIYNQKFKGKATLTVDKSSSTAYMELRSLTSEDIAVYYCAREGRGGAWFDSWGQGTLVTVSAASTKGPSVFPLAPSSKSTSGGTAALGCLVKDYFPEPVTVSWNSGALTSGVHTFPAVLQSSGLYSLSSVVTVPSSSLGTQTYICNVNHKPSNTKVDKKVEPKSCDKTHTCPPCPAPEAAGAPSVFLFPPKPKDTLMISRTPEVTCVVVDVSHEDPEVKFNWYVDGVEVHNAKTKPREEQYNSTYRVVSVLTVLHQDWLNGKEYKCKVSNKALPAPIEKTISKAKGQPREPQVYTLPPSREEMTKNQVSLTCLVKGFYPSDIAVEWESNGQPENNYKTTPPVLDSDGSFFLYSKLTVDKSRWQQGNVFSCSVMHEALHNHYTQKSLSLSPG

SEQ ID NO: 169 - protein, 447 aa, synthetic construct; identical to SEQ ID NO: 156

SEQ ID NO: 170 - protein, 447 aa, synthetic construct; identical to SEQ ID NO: 151

SEQ ID NO: 171 - protein, 447 aa, synthetic construct
QVQLQESGPGLVKPSETLSLTCTFSGFSLSTYGIGVGWIRQPPGKGLEWIAHIWWNNNKYFNTALKSRLTISKDTSKNQVSLKLSSVTAADTAVYYCARMGYDIMDYWGQGTLVTVSSASTKGPSVFPLAPSSKSTSGGTAALGCLVKDYFPEPVTVSWNSGALTSGVHTFPAVLQSSGLYSLSSVVTVPSSSLGTQTYICNVNHKPSNTKVDKKVEPKSCDKTHTCPPCPAPEAAGAPSVFLFPPKPKDTLMISRTPEVTCVVVDVSHEDPEVKFNWYVDGVEVHNAKTKPREEQYNSTYRVVSVLTVLHQDWLNGKEYKCKVSNKALPAPIEKTISKAKGQPREPQVYTLPPSREEMTKNQVSLTCLVKGFYPSDIAVEWESNGQPENNYKTTPPVLDSDGSFFLYSKLTVDKSRWQQGNVFSCSVMHEALHNHYTQKSLSLSPG

SEQ ID NO: 172 - protein, 447 aa, synthetic construct
QVTLQESGPGLVKPSETLSLTCSFSGFSLSTYGIGVGWIRQPPGKGLEWLAHIWWNNNKYFNTALKSRLTISKDTSKNQVSLKLSSVTAADTATYYCARMGYDIMDYWGQGTSVTVSSASTKGPSVFPLAPSSKSTSGGTAALGCLVKDYFPEPVTVSWNSGALTSGVHTFPAVLQSSGLYSLSSVVTVPSSSLGTQTYICNVNHKPSNTKVDKKVEPKSCDKTHTCPPCPAPEAAGAPSVFLFPPKPKDTLMISRTPEVTCVVVDVSHEDPEVKFNWYVDGVEVHNAKTKPREEQYNSTYRVVSVLTVLHQDWLNGKEYKCKVSNKALPAPIEKTISKAKGQPREPQVYTLPPSREEMTKNQVSLTCLVKGFYPSDIAVEWESNGQPENNYKTTPPVLDSDGSFFLYSKLTVDKSRWQQGNVFSCSVMHEALHNHYTQKSLSLSPG

SEQ ID NO: 173 - protein, 447 aa, synthetic construct
EVQLLESGGGLVQPGGSLRLSCAFSGFSLSTYGIGVGWIRQAPGKGLEWVAHIWWNNNKYFNTALKSRLTISKDTSKNTVYLQMNSLRAEDTAVYYCAKMGYDIMDYWGQGTTVTVSSASTKGPSVFPLAPSSKSTSGGTAALGCLVKDYFPEPVTVSWNSGALTSGVHTFPAVLQSSGLYSLSSVVTVPSSSLGTQTYICNVNHKPSNTKVDKKVEPKSCDKTHTCPPCPAPEAAGAPSVFLFPPKPKDTLMISRTPEVTCVVVDVSHEDPEVKFNWYVDGVEVHNAKTKPREEQYNSTYRVVSVLTVLHQDWLNGKEYKCKVSNKALPAPIEKTISKAKGQPREPQVYTLPPSREEMTKNQVSLTCLVKGFYPSDIAVEWESNGQPENNYKTTPPVLDSDGSFFLYSKLTVDKSRWQQGNVFSCSVMHEALHNHYTQKSLSLSPG

SEQ ID NO: 174 - protein, 447 aa, synthetic construct
QVTLLESGGGLVQPGGSLRLSCSFSGFSLSTYGIGVGWIRQAPGKGLEWLAHIWWNNNKYFNTALKSRLTISKDTSKNTVYLQMNSVRAEDTAVYYCARMGYDIMDYWGQGTTVTVSSASTKGPSVFPLAPSSKSTSGGTAALGCLVKDYFPEPVTVSWNSGALTSGVHTFPAVLQSSGLYSLSSVVTVPSSSLGTQTYICNVNHKPSNTKVDKKVEPKSCDKTHTCPPCPAPEAAGAPSVFLFPPKPKDTLMISRTPEVTCVVVDVSHEDPEVKFNWYVDGVEVHNAKTKPREEQYNSTYRVVSVLTVLHQDWLNGKEYKCKVSNKALPAPIEKTISKAKGQPREPQVYTLPPSREEMTKNQVSLTCLVKGFYPSDIAVEWESNGQPENNYKTTPPVLDSDGSFFLYSKLTVDKSRWQQGNVFSCSVMHEALHNHYTQKSLSLSPG

SEQ ID NO: 175 - protein, 448 aa, synthetic construct
EVQLVQSGAEVKKPGASVKVSCKASGYTFTDYNLNWVRQATGQGLEWMGDLNPYNQGIIYNQKFKGRVTMTVDTSISTAYMELSSLRSEDTAVYYCAREGRGGAWFDSWGQGTLVTVSSASTKGPSVFPLAPSSKSTSGGTAALGCLVKDYFPEPVTVSWNSGALTSGVHTFPAVLQSSGLYSLSSVVTVPSSSLGTQTYICNVNHKPSNTKVDKKVEPKSCDKTHTCPPCPAPEAAGAPSVFLFPPKPKDTLMISRTPEVTCVVVDVSHEDPEVKFNWYVDGVEVHNAKTKPREEQYNSTYRVVSVLTVLHQDWLNGKEYKCKVSNKALPAPIEKTISKAKGQPREPQVYTLPPSREEMTKNQVSLTCLVKGFYPSDIAVEWESNGQPENNYKTTPPVLDSDGSFFLYSKLTVDKSRWQQGNVFSCSVMHEALHNHYTQKSLSLSPG

SEQ ID NO: 176 - protein, 448 aa, synthetic construct
EVQLVQSGAEVKKPGASVKVSCKASGYTFTDYNLNWVRQATGQGLEWMGDLNPYNQGIIYNQKFKGRVTLTVDKSISTAYMELSSLRSEDTAVYYCAREGRGGAWFDSWGQGTLVTVSSASTKGPSVFPLAPSSKSTSGGTAALGCLVKDYFPEPVTVSWNSGALTSGVHTFPAVLQSSGLYSLSSVVTVPSSSLGTQTYICNVNHKPSNTKVDKKVEPKSCDKTHTCPPCPAPEAAGAPSVFLFPPKPKDTLMISRTPEVTCVVVDVSHEDPEVKFNWYVDGVEVHNAKTKPREEQYNSTYRVVSVLTVLHQDWLNGKEYKCKVSNKALPAPIEKTISKAKGQPREPQVYTLPPSREEMTKNQVSLTCLVKGFYPSDIAVEWESNGQPENNYKTTPPVLDSDGSFFLYSKLTVDKSRWQQGNVFSCSVMHEALHNHYTQKSLSLSPG

SEQ ID NO: 177 - protein, 448 aa, synthetic construct
EVQLVQSGAEVKKPGASVKVSCKASGYTFTDYNLNWVRQATGQGLEWIGDLNPYNQGIIYNQKFKGRATLTVDKSISTAYMELSSLRSEDTAVYYCAREGRGGAWFDSWGQGTLVTVSSASTKGPSVFPLAPSSKSTSGGTAALGCLVKDYFPEPVTVSWNSGALTSGVHTFPAVLQSSGLYSLSSVVTVPSSSLGTQTYICNVNHKPSNTKVDKKVEPKSCDKTHTCPPCPAPEAAGAPSVFLFPPKPKDTLMISRTPEVTCVVVDVSHEDPEVKFNWYVDGVEVHNAKTKPREEQYNSTYRVVSVLTVLHQDWLNGKEYKCKVSNKALPAPIEKTISKAKGQPREPQVYTLPPSREEMTKNQVSLTCLVKGFYPSDIAVEWESNGQPENNYKTTPPVLDSDGSFFLYSKLTVDKSRWQQGNVFSCSVMHEALHNHYTQKSLSLSPG

SEQ ID NO: 178 - protein, 448 aa, synthetic construct
EVQLVQSGAEVKKPGASVKVSCKASGYTLTDYNLNWVRQATGQGLEWIGDLNPYNQGIIYNQKFKGRATLTVNKSISTAYMELSSLRSEDTAVYYCAREGRGGAWFDSWGQGTLVTVSSASTKGPSVFPLAPSSKSTSGGTAALGCLVKDYFPEPVTVSWNSGALTSGVHTFPAVLQSSGLYSLSSVVTVPSSSLGTQTYICNVNHKPSNTKVDKKVEPKSCDKTHTCPPCPAPEAAGAPSVFLFPPKPKDTLMISRTPEVTCVVVDVSHEDPEVKFNWYVDGVEVHNAKTKPREEQYNSTYRVVSVLTVLHQDWLNGKEYKCKVSNKALPAPIEKTISKAKGQPREPQVYTLPPSREEMTKNQVSLTCLVKGFYPSDIAVEWESNGQPENNYKTTPPVLDSDGSFFLYSKLTVDKSRWQQGNVFSCSVMHEALHNHYTQKSLSLSPG

SEQ ID NO: 179 - protein, 447 aa, synthetic construct
QVTLKESGPALVKPTQTLTLTCTFSGFSLSTYGIGVGWIRQPPGKALEWLAHIWWNDNKYYNTALKSRLTISKDTSKNQVVLTMTNMDPVDTATYYCARLAYDYVDSWGQGTTLTVSSASTKGPSVFPLAPSSKSTSGGTAALGCLVKDYFPEPVTVSWNSGALTSGVHTFPAVLQSSGLYSLSSVVTVPSSSLGTQTYICNVNHKPSNTKVDKKVEPKSCDKTHTCPPCPAPEAAGAPSVFLFPPKPKDTLMISRTPEVTCVVVDVSHEDPEVKFNWYVDGVEVHNAKTKPREEQYNSTYRVVSVLTVLHQDWLNGKEYKCKVSNKALPAPIEKTISKAKGQPREPQVYTLPPSREEMTKNQVSLTCLVKGFYPSDIAVEWESNGQPENNYKTTPPVLDSDGSFFLYSKLTVDKSRWQQGNVFSCSVMHEALHNHYTQKSLSLSPG

SEQ ID NO: 180 - protein, 447 aa, synthetic construct
QVTLKESGPALVKPTQTLTLTCTFSGFSLSTYGIGVGWIRQPPGKGLEWLAHIWWNDNKYYNTALKSRLTISKDTSKNQVVLTMTNMDPVDTATYYCARLAYDYVDSWGQGTTLTVSSASTKGPSVFPLAPSSKSTSGGTAALGCLVKDYFPEPVTVSWNSGALTSGVHTFPAVLQSSGLYSLSSVVTVPSSSLGTQTYICNVNHKPSNTKVDKKVEPKSCDKTHTCPPCPAPEAAGAPSVFLFPPKPKDTLMISRTPEVTCVVVDVSHEDPEVKFNWYVDGVEVHNAKTKPREEQYNSTYRVVSVLTVLHQDWLNGKEYKCKVSNKALPAPIEKTISKAKGQPREPQVYTLPPSREEMTKNQVSLTCLVKGFYPSDIAVEWESNGQPENNYKTTPPVLDSDGSFFLYSKLTVDKSRWQQGNVFSCSVMHEALHNHYTQKSLSLSPG

SEQ ID NO: 181 - protein, 447 aa, synthetic construct
QITLKESGPTLVKPTQTLTLTCTFSGFSLSTYGIGVGWIRQPPGKALEWLAHIWWNDNKYYNTALKSRLTITKDTSKNQVVLTMTNMDPVDTATYYCARLAYDYVDSWGQGTLVTVSSASTKGPSVFPLAPSSKSTSGGTAALGCLVKDYFPEPVTVSWNSGALTSGVHTFPAVLQSSGLYSLSSVVTVPSSSLGTQTYICNVNHKPSNTKVDKKVEPKSCDKTHTCPPCPAPEAAGAPSVFLFPPKPKDTLMISRTPEVTCVVVDVSHEDPEVKFNWYVDGVEVHNAKTKPREEQYNSTYRVVSVLTVLHQDWLNGKEYKCKVSNKALPAPIEKTISKAKGQPREPQVYTLPPSREEMTKNQVSLTCLVKGFYPSDIAVEWESNGQPENNYKTTPPVLDSDGSFFLYSKLTVDKSRWQQGNVFSCSVMHEALHNHYTQKSLSLSPG

SEQ ID NO: 182 - protein, 447 aa, synthetic construct
QITLKESGPALVKPTQTLTLTCTFSGFSLSTYGIGVGWIRQPPGKALEWLAHIWWNDNKYYNTALKSRLTITKDTSKNQVFLTMTNMDPVDTATYYCARLAYDYVDSWGQGTLVTVSSASTKGPSVFPLAPSSKSTSGGTAALGCLVKDYFPEPVTVSWNSGALTSGVHTFPAVLQSSGLYSLSSVVTVPSSSLGTQTYICNVNHKPSNTKVDKKVEPKSCDKTHTCPPCPAPEAAGAPSVFLFPPKPKDTLMISRTPEVTCVVVDVSHEDPEVKFNWYVDGVEVHNAKTKPREEQYNSTYRVVSVLTVLHQDWLNGKEYKCKVSNKALPAPIEKTISKAKGQPREPQVYTLPPSREEMTKNQVSLTCLVKGFYPSDIAVEWESNGQPENNYKTTPPVLDSDGSFFLYSKLTVDKSRWQQGNVFSCSVMHEALHNHYTQKSLSLSPG

SEQ ID NO: 183 - protein, 214 aa, synthetic construct
DIVMTQSHKFMSTSVGDRVSITCKASQDVNTAVAWYQQKPGQSPKFLIYSSSYRYTGVPDRFTGSGSGTDFTFTISSVQAEDLAVYYCQQHYSTPWTFGGGTKLEIKRTVAAPSVFIFPPSDEQLKSGTASVVCLLNNFYPREAKVQWKVDNALQSGNSQESVTEQDSKDSTYSLSSTLTLSKADYEKHKVYACEVTHQGLSSPVTKSFNRGEC

SEQ ID NO: 184 - protein, 214 aa, synthetic construct
DIVMTQSQKFMSTSVGDRVSVTCKASQNVGTNVAWYQQKPGQSPKGLIYSASYRYSGVPDRFTGSGSGTDFTLTISNVQSEDLAEYFCQQYNSYPWTFGGGTKLEIKRTVAAPSVFIFPPSDEQLKSGTASVVCLLNNFYPREAKVQWKVDNALQSGNSQESVTEQDSKDSTYSLSSTLTLSKADYEKHKVYACEVTHQGLSSPVTKSFNRGEC

SEQ ID NO: 185 - protein, 214 aa, synthetic construct
DIVMTQSQKFMSTSVGDRVSVTCKASQNVGTNVAWYQQKPGQSPKGLIYSASYRYSGVPDRFTGSGSGTDFTLTINNVQSEDLAEYFCQQYNSYPYTFGGGTKLEIKRTVAAPSVFIFPPSDEQLKSGTASVVCLLNNFYPREAKVQWKVDNALQSGNSQESVTEQDSKDSTYSLSSTLTLSKADYEKHKVYACEVTHQGLSSPVTKSFNRGEC

SEQ ID NO: 186 - protein, 214 aa, synthetic construct
DIQMTQSSSSFSVSLGDRVTITCKASEDIYHRLAWYQQKPGNAPRLLISGATSLETGIPSRFSGSGSGKDYALSITSLQTEDVGTYYCQQYWSPPFTFGSGTKLEIKRTVAAPSVFIFPPSDEQLKSGTASVVCLLNNFYPREAKVQWKVDNALQSGNSQESVTEQDSKDSTYSLSSTLTLSKADYEKHKVYACEVTHQGLSSPVTKSFNRGEC

SEQ ID NO: 187 - protein, 214 aa, synthetic construct
DIQMTQSPASLSVSVGETVTITCRPSESIYSNLAWYQQKQGKSPQLLVYAATNLADGVPSRFSGSGSGTQYSLKINSLQSEDFGTYYCQHFWGIPWTFGGGTKLEIKRTVAAPSVFIFPPSDEQLKSGTASVVCLLNNFYPREAKVQWKVDNALQSGNSQESVTEQDSKDSTYSLSSTLTLSKADYEKHKVYACEVTHQGLSSPVTKSFNRGEC

SEQ ID NO: 188 - protein, 214 aa, synthetic construct
DIQMTQSPASLSVSVGETVTITCRASENIYSNLAWYQQKQGKSPQLLVYAATNLGDGAPSRFSGSGSGTQYSLKINSLQSEDFGSYYCQHFWGTPWTFGGGTKLEIKRTVAAPSVFIFPPSDEQLKSGTASVVCLLNNFYPREAKVQWKVDNALQSGNSQESVTEQDSKDSTYSLSSTLTLSKADYEKHKVYACEVTHQGLSSPVTKSFNRGEC

SEQ ID NO: 189 - protein, 219 aa, synthetic construct
DIVMTQAAFSNPVTLGTSASISCRSSKSLLHSNGITYLYWYLQKPGQSPQLLIYQMSNLVSGVPDRFSSSGSGTDFTLRISRVEAEDVGVYYCAQNLELPPTFGAGTKLELKRTVAAPSVFIFPPSDEQLKSGTASVVCLLNNFYPREAKVQWKVDNALQSGNSQESVTEQDSKDSTYSLSSTLTLSKADYEKHKVYACEVTHQGLSSPVTKSFNRGEC

SEQ ID NO: 190 - protein, 214 aa, synthetic construct
DIQMTQSPASLSVSVGETVTITCRASENIYSNLAWYQQKQGKSPQLLVSAATNLADGVPSRFSGSGSGTQYSLKIISLQSVDFGSYYCQHFWGTPWTFGGGTKLEIKRTVAAPSVFIFPPSDEQLKSGTASVVCLLNNFYPREAKVQWKVDNALQSGNSQESVTEQDSKDSTYSLSSTLTLSKADYEKHKVYACEVTHQGLSSPVTKSFNRGEC

SEQ ID NO: 191 - protein, 214 aa, synthetic construct
DIQMTQTTSSLSASLGDRVTISCRASQDISNYLNWYQQKPDGTVKLLIHSASNLHSGVPSRFSGSGSGTDYSLTISNLEQEDIATYFCQQYNMFPWTFGGGTKLEIKRTVAAPSVFIFPPSDEQLKSGTASVVCLLNNFYPREAKVQWKVDNALQSGNSQESVTEQDSKDSTYSLSSTLTLSKADYEKHKVYACEVTHQGLSSPVTKSFNRGEC

SEQ ID NO: 192 - protein, 214 aa, synthetic construct
DNKMTQSPSSMYASLGERVTITCKASQDINSYLSWFQQKPGKSPKTLIYRANKLVDGVPSRFSGSGSGQDYSLTISSLEYEDMGIYHCLQYDEFPYTFGGGTKLEIKRTVAAPSVFIFPPSDEQLKSGTASVVCLLNNFYPREAKVQWKVDNALQSGNSQESVTEQDSKDSTYSLSSTLTLSKADYEKHKVYACEVTHQGLSSPVTKSFNRGEC

SEQ ID NO: 193 - protein, 213 aa, synthetic construct
DIQMTQSPASLSVSVGETVTITCRASENIYSNLAWYQQKQGKSPQLLVYAATDLADGVPSRFSGSGSGTQYSLKINSLQSEDFGNYHCQLFWGTPTFGGGTKLEIKRTVAAPSVFIFPPSDEQLKSGTASVVCLLNNFYPREAKVQWKVDNALQSGNSQESVTEQDSKDSTYSLSSTLTLSKADYEKHKVYACEVTHQGLSSPVTKSFNRGEC

SEQ ID NO: 194 - protein, 215 aa, synthetic construct
EIVLTQSPALMAASPGEKVTITCSVSSSISSSNLHWYQQKSETSPKPWIYGTSNLASGVPVRFSGSGSGTSYSLTISSMEAEDAATYYCQQWSSYPLTFGAGTKLELKRTVAAPSVFIFPPSDEQLKSGTASVVCLLNNFYPREAKVQWKVDNALQSGNSQESVTEQDSKDSTYSLSSTLTLSKADYEKHKVYACEVTHQGLSSPVTKSFNRGEC

SEQ ID NO: 195 - protein, 214 aa, synthetic construct
DIVMTQSQKFMSTSVGDRVSVTCKASQNVGTNIAWFQQKPGQSPEALIYSASYRYSGVPDRFTGSGSGTDFTLTISNVQSEDLAEYFCQQYNTYPHTFGGGTKLEIRRTVAAPSVFIFPPSDEQLKSGTASVVCLLNNFYPREAKVQWKVDNALQSGNSQESVTEQDSKDSTYSLSSTLTLSKADYEKHKVYACEVTHQGLSSPVTKSFNRGEC

SEQ ID NO: 196 - protein, 214 aa, synthetic construct
DIVMTQSQKFMSTSVGDRVSVTCKASQNVGSNVAWYQQKPGQSPKALIYSASYRYSGVPDRFTGSGSGTDFTLTITNVQSEDLAEYFCQQYKSYPLTFGAGTKLELKRTVAAPSVFIFPPSDEQLKSGTASVVCLLNNFYPREAKVQWKVDNALQSGNSQESVTEQDSKDSTYSLSSTLTLSKADYEKHKVYACEVTHQGLSSPVTKSFNRGEC

SEQ ID NO: 197 - protein, 214 aa, synthetic construct
ETTVTQSPASLSMAIGEKVTIRCITSIDIDDDINWYQQKPGEPPNLLISEGNTLRPGVPSRFSSSGYGTDFVFTIENMLSEDVADYYCLQSDNLPLTFGGGTKLEIKRTVAAPSVFIFPPSDEQLKSGTASVVCLLNNFYPREAKVQWKVDNALQSGNSQESVTEQDSKDSTYSLSSTLTLSKADYEKHKVYACEVTHQGLSSPVTKSFNRGEC

SEQ ID NO: 198 - skipped

SEQ ID NO: 199 - protein, 214 aa, synthetic construct; identical to SEQ ID NO: 186

SEQ ID NO: 200 - protein, 219 aa, synthetic construct
DIVMTQAAFSNPVTLGTSASISCRSSKSLLHSNAITYLYWYLQKPGQSPQLLIYQMSNLVSGVPDRFSSSGSGTDFTLRISRVEAEDVGVYYCAQNLELPPTFGAGTKLELKRTVAAPSVFIFPPSDEQLKSGTASVVCLLNNFYPREAKVQWKVDNALQSGNSQESVTEQDSKDSTYSLSSTLTLSKADYEKHKVYACEVTHQGLSSPVTKSFNRGEC

SEQ ID NO: 201 - protein, 219 aa, synthetic construct
DIVMTQAAFSNPVTLGTSASISCRSSKSLLHSNQITYLYWYLQKPGQSPQLLIYQMSNLVSGVPDRFSSSGSGTDFTLRISRVEAEDVGVYYCAQNLELPPTFGAGTKLELKRTVAAPSVFIFPPSDEQLKSGTASVVCLLNNFYPREAKVQWKVDNALQSGNSQESVTEQDSKDSTYSLSSTLTLSKADYEKHKVYACEVTHQGLSSPVTKSFNRGEC

SEQ ID NO: 202 - protein, 219 aa, synthetic construct
DIVMTQAAFSNPVTLGTSASISCRSSKSLLHSEGITYLYWYLQKPGQSPQLLIYQMSNLVSGVPDRFSSSGSGTDFTLRISRVEAEDVGVYYCAQNLELPPTFGAGTKLELKRTVAAPSVFIFPPSDEQLKSGTASVVCLLNNFYPREAKVQWKVDNALQSGNSQESVTEQDSKDSTYSLSSTLTLSKADYEKHKVYACEVTHQGLSSPVTKSFNRGEC

SEQ ID NO: 203 - protein, 214 aa, synthetic construct
DIVMTQSQKFMSTSVGDRVSVTCKASQNVGTNVAWYQQKPGQSPKGLIYSASYRYSGVPDRFTGSGSGTDFTLTISNVQSEDLAEYFCQQYNAYPWTFGGGTKLEIKRTVAAPSVFIFPPSDEQLKSGTASVVCLLNNFYPREAKVQWKVDNALQSGNSQESVTEQDSKDSTYSLSSTLTLSKADYEKHKVYACEVTHQGLSSPVTKSFNRGEC

SEQ ID NO: 204 - protein, 214 aa, synthetic construct
DIVMTQSQKFMSTSVGDRVSVTCKASQNVGTNVAWYQQKPGQSPKGLIYSASYRYSGVPDRFTGSGSGTDFTLTISNVQSEDLAEYFCQQYESYPWTFGGGTKLEIKRTVAAPSVFIFPPSDEQLKSGTASVVCLLNNFYPREAKVQWKVDNALQSGNSQESVTEQDSKDSTYSLSSTLTLSKADYEKHKVYACEVTHQGLSSPVTKSFNRGEC

SEQ ID NO: 205 - protein, 214 aa, synthetic construct
DIVMTQSQKFMSTSVGDRVSVTCKASQNVGTNVAWYQQKPGQSPKGLIYSASYRYSGVPDRFTGSGSGTDFTLTISNVQSEDLAEYFCQQYNQYPWTFGGGTKLEIKRTVAAPSVFIFPPSDEQLKSGTASVVCLLNNFYPREAKVQWKVDNALQSGNSQESVTEQDSKDSTYSLSSTLTLSKADYEKHKVYACEVTHQGLSSPVTKSFNRGEC

SEQ ID NO: 206 - protein, 214 aa, synthetic construct
DIQMTQSPSSLSTSVGDRVTITCKASQDVNTAVAWYQQKPGKAPKFLIYSSSYRYTGVPDRFSGSGSGTDFTFTISSLQPEDFAVYYCQQHYSTPWTFGQGTKVEIKRTVAAPSVFIFPPSDEQLKSGTASVVCLLNNFYPREAKVQWKVDNALQSGNSQESVTEQDSKDSTYSLSSTLTLSKADYEKHKVYACEVTHQGLSSPVTKSFNRGEC

SEQ ID NO: 207 - protein, 214 aa, synthetic construct
DIVMTQSPSSLSTSVGDRVTITCKASQDVNTAVAWYQQKPGKSPKFLIYSSSYRYTGVPDRFSGSGSGTDFTFTISSVQPEDFAVYYCQQHYSTPWTFGGGTKVEIKRTVAAPSVFIFPPSDEQLKSGTASVVCLLNNFYPREAKVQWKVDNALQSGNSQESVTEQDSKDSTYSLSSTLTLSKADYEKHKVYACEVTHQGLSSPVTKSFNRGEC

SEQ ID NO: 208 - protein, 214 aa, synthetic construct
DIVMTQSPATLSTSPGERATLSCKASQDVNTAVAWYQQKPGQAPRFLIYSSSYRYTGVPARFSGSGSGTEFTFTISSLQSEDFAVYYCQQHYSTPWTFGGGTKVEIKRTVAAPSVFIFPPSDEQLKSGTASVVCLLNNFYPREAKVQWKVDNALQSGNSQESVTEQDSKDSTYSLSSTLTLSKADYEKHKVYACEVTHQGLSSPVTKSFNRGEC

SEQ ID NO: 209 - protein, 214 aa, synthetic construct
DIVMTQSPATLSTSPGERVTISCKASQDVNTAVAWYQQKPGQSPRFLIYSSSYRYTGVPDRFSGSGSGTDFTFTISSVQSEDFAVYYCQQHYSTPWTFGGGTKVEIKRTVAAPSVFIFPPSDEQLKSGTASVVCLLNNFYPREAKVQWKVDNALQSGNSQESVTEQDSKDSTYSLSSTLTLSKADYEKHKVYACEVTHQGLSSPVTKSFNRGEC

SEQ ID NO: 210 - protein, 214 aa, synthetic construct
DIQMTQSPSSLSASVGDRVTITCKASEDIYHRLAWYQQKPGKAPKLLIYGATSLETGVPSRFSGSGSGTDFTFTISSLQPEDIATYYCQQYWSPPFTFGGGTKVEIKRTVAAPSVFIFPPSDEQLKSGTASVVCLLNNFYPREAKVQWKVDNALQSGNSQESVTEQDSKDSTYSLSSTLTLSKADYEKHKVYACEVTHQGLSSPVTKSFNRGEC

SEQ ID NO: 211 - protein, 214 aa, synthetic construct
DIQMTQSPSSLSASVGDRVTITCKASEDIYHRLAWYQQKPGKAPKLLIYGATSLETGVPSRFSGSGSGTDYTFTISSLQPEDIATYYCQQYWSPPFTFGGGTKVEIKRTVAAPSVFIFPPSDEQLKSGTASVVCLLNNFYPREAKVQWKVDNALQSGNSQESVTEQDSKDSTYSLSSTLTLSKADYEKHKVYACEVTHQGLSSPVTKSFNRGEC

SEQ ID NO: 212 - protein, 214 aa, synthetic construct
DIQMTQSPSSLSASVGDRVTITCKASEDIYHRLAWYQQKPGKAPKLLISGATSLETGVPSRFSGSGSGTDYTFTISSLQPEDIATYYCQQYWSPPFTFGGGTKVEIKRTVAAPSVFIFPPSDEQLKSGTASVVCLLNNFYPREAKVQWKVDNALQSGNSQESVTEQDSKDSTYSLSSTLTLSKADYEKHKVYACEVTHQGLSSPVTKSFNRGEC

SEQ ID NO: 213 - protein, 214 aa, synthetic construct
DIQMTQSPSSLSASVGDRVTITCKASEDIYHRLAWYQQKPGKAPKLLISGATSLETGIPSRFSGSGSGTDYTFTISSLQPEDIATYYCQQYWSPPFTFGGGTKVEIKRTVAAPSVFIFPPSDEQLKSGTASVVCLLNNFYPREAKVQWKVDNALQSGNSQESVTEQDSKDSTYSLSSTLTLSKADYEKHKVYACEVTHQGLSSPVTKSFNRGEC

SEQ ID NO: 214 - protein, 219 aa, synthetic construct
DIVMTQTPLSLSVTPGQPASISCRSSKSLLHSEGITYLYWYLQKPGQSPQLLIYQMSNLVSGVPDRFSGSGSGTDFTLKISRVEAEDVGVYYCAQNLELPPTFGQGTKLEIKRTVAAPSVFIFPPSDEQLKSGTASVVCLLNNFYPREAKVQWKVDNALQSGNSQESVTEQDSKDSTYSLSSTLTLSKADYEKHKVYACEVTHQGLSSPVTKSFNRGEC

SEQ ID NO: 215 - protein, 219 aa, synthetic construct
DIVMTQTPLSLSVTPGQPASISCRSSKSLLHSEGITYLYWYLQKPGQSPQLLIYQMSNLVSGVPDRFSSSGSGTDFTLKISRVEAEDVGVYYCAQNLELPPTFGQGTKLEIKRTVAAPSVFIFPPSDEQLKSGTASVVCLLNNFYPREAKVQWKVDNALQSGNSQESVTEQDSKDSTYSLSSTLTLSKADYEKHKVYACEVTHQGLSSPVTKSFNRGEC

SEQ ID NO: 216 - protein, 219 aa, synthetic construct
DIVMTQTPLSLSVTPGQPASISCKSSKSLLHSEGITYLYWYLQKPGQSPQLLIYQMSNLVSGVPDRFSGSGSGTDFTLKISRVEAEDVGVYYCAQNLELPPTFGQGTKLEIKRTVAAPSVFIFPPSDEQLKSGTASVVCLLNNFYPREAKVQWKVDNALQSGNSQESVTEQDSKDSTYSLSSTLTLSKADYEKHKVYACEVTHQGLSSPVTKSFNRGEC

SEQ ID NO: 217 - protein, 219 aa, synthetic construct
DIVMTQSPLSLSVTPGEPASISCRSSKSLLHSEGITYLYWYLQKPGQSPQLLIYQMSNLVSGVPDRFSGSGSGTDFTLKISRVEAEDVGVYYCAQNLELPPTFGQGTKLEIKRTVAAPSVFIFPPSDEQLKSGTASVVCLLNNFYPREAKVQWKVDNALQSGNSQESVTEQDSKDSTYSLSSTLTLSKADYEKHKVYACEVTHQGLSSPVTKSFNRGEC

SEQ ID NO: 218 - protein, 120 aa, synthetic construct
EVLLQQSGPELVKPGASVKIPCKASGYTFTDYNMDWVKQSHGKSLEWIGQINPNNGGIFFNQKFKGKATLTVDKSSNTAFMEVRSLTSEDTAVYYCAREAITTVGAMDYWGQGTSVTVSS

SEQ ID NO: 219 - protein, 107 aa, synthetic construct
DIQMTQSPASLSASVGETVTITCRTSENLHNYLAWYQQKQGKSPQLLVYDAKTLADGVPSRFSGSGSGTQYSLKINSLQPEDFGSYYCQHFWSSPYTFGGGTKLEIK

SEQ ID NO: 220 - protein, 120 aa, synthetic construct
QVQLVQSGAEVKKPGSSVKVSCKASGYTFSSYNIDWVRQAPGQGLEWMGGINPIFGTAFYNQKFQGRVTITADESTSTAYMELSSLRSEDTAVYYCAREAITTVGAMDHWGQGTLVTVSS

SEQ ID NO: 221 - protein, 107 aa, synthetic construct
EIVLTQSPATLSLSPGERATLSCRTSQSVHNYLAWYQQKPGQAPRLLIYDASTRADGIPARFSGSGSGTDFTLTISSLEPEDFAVYYCQQFWSWPWTFGQGTKVEIK

SEQ ID NO: 222 - protein, 116 aa, synthetic construct
DVQLQESGPGLVKPSQSLSLTCTVTGYSITSAYAWNWIRQFPGNKLEWMGYISYSGSTSYNPSLKSRISITRDTSKNQFFLQFNSVTTEDTATYYCARGGDAEDYWGQGTTLTVSS

SEQ ID NO: 223 - protein, 107 aa, synthetic construct
DIQMTQSPASLSVSVGETVTITCRASENIYSNLAWFQQKQGKSPQLLVYVATNLVDGVPSRFSGSGSGTQYSLKINSLQSEDFGTYYCQHFWGTPWTFGGGTKLEIK

SEQ ID NO: 224 - protein, 118 aa, synthetic construct
QITLKESGPTLVKPTQTLTLTCTFSGFSLSTSGMGVSWIRQPPGKGLEWLAHIYWDDDKRYNPTLKSRLTITKDPSKNQVVLTMTNMDPVDTATYYCARSSYGAMDYWGQGTLVTVSS

SEQ ID NO: 225 - protein, 107 aa, synthetic construct
DIVLTQSPSFLSASVGDRVTITCKASQNVGTNVAWFQQKPGKSPKALIYSASYRYSGVPDRFTGSGSGTEFTLTISSLQPEDFAAYFCQQYNNFPYTFGGGTKLEIK

SEQ ID NO: 226 - protein, 112 aa, synthetic construct
EVQLQQSGAELVRPGALVKLSCKASGFNIKDYYMHWVRQRPEQGLEWIGWIDPENGNTIYDPKFQGKASITTDTSSNTAYMQLSSLTCEDTAVYYCAVPDSWGQGTTLTVSS

SEQ ID NO: 227 - protein, 112 aa, synthetic construct
DIVMTQAAPSVPVTPGESVSISCRSSKSLLHSNGNTYLYWFLQRPDQSPQLLIYRMSNLASGVPDRFSGSGSGTAFTLRISRVEAEDVGVYYCMQHLEYPFTFGSGTKLEIK

SEQ ID NO: 228 - protein, 329 aa, synthetic construct
ASTKGPSVFPLAPSSKSTSGGTAALGCLVKDYFPEPVTVSWNSGALTSGVHTFPAVLQSSGLYSLSSVVTVPSSSLGTQTYICNVNHKPSNTKVDKRVEPKSCDKTHTCPPCPAPEAAGAPSVFLFPPKPKDTLMISRTPEVTCVVVDVSHEDPEVKFNWYVDGVEVHNAKTKPREEQYNSTYRVVSVLTVLHQDWLNGKEYKCKVSNKALPAPIEKTISKAKGQPREPQVYTLPPSRDELTKNQVSLTCLVKGFYPSDIAVEWESNGQPENNYKTTPPVLDSDGSFFLYSKLTVDKSRWQQGNVFSCSVMHEALHNHYTQKSLSLSPG

SEQ ID NO: 229 - protein, 447 aa, synthetic construct
QITLKESGPTLVKPTQTLTLTCTFSGFSLSTYGIGVGWIRQPPGKALEWLAHIWWNDNKYYNTALKSRLTITKDTSKNQVVLTMTNMDPVDTATYYCARLAYDYVDSWGQGTLVTVSSASTKGPSVFPLAPSSKSTSGGTAALGCLVKDYFPEPVTVSWNSGALTSGVHTFPAVLQSSGLYSLSSVVTVPSSSLGTQTYICNVNHKPSNTKVDKRVEPKSCDKTHTCPPCPAPEAAGAPSVFLFPPKPKDTLMISRTPEVTCVVVDVSHEDPEVKFNWYVDGVEVHNAKTKPREEQYNSTYRVVSVLTVLHQDWLNGKEYKCKVSNKALPAPIEKTISKAKGQPREPQVYTLPPSRDELTKNQVSLTCLVKGFYPSDIAVEWESNGQPENNYKTTPPVLDSDGSFFLYSKLTVDKSRWQQGNVFSCSVMHEALHNHYTQKSLSLSPG